European Patent Specification EP 3 731 855 B1, published July 23, 2025. Title: Immunogenic sequences from a Phage Tail Length Tape Measure Protein, bacteria expressing the same and their use in treating a cancer. Applicant: Institut Gustave Roussy. The sequence listing filed with the application follows.

SEQUENCE LISTING (211 sequences)

SEQ ID NO: 1 - protein, 1506 aa, Enterococcus hirae
MAQSKTVKAVLTAIDKGFTQTMGSATSSLKKLSSNASDIPSNLNTVSGAMKSFGDKTASIGQSIEKVGGSMTKGITLPIAGAVGAVTTAAVKWESAFTGVKKTNDEMVDSNGKVIYSYDDLEKGLRDLAKELPTSHEEIAKVAEAAGQLGIKTDKVVGFTKTMIDMGESTNMSADTAATSLARFANITQMSQDKFSNLGSAIVDLGNNLATTESEITEMGLRLAGAGKQIGMTEGDIVGFAAALSSVGIEAEAGGSAFSRLMVQMQLATETGVKAFEPLKQAVAIQGVSWEKFVHAVNWGGKELTAVSKQMGVPASELKKLYKEASKASGSLEDFANVTGRTGEEFAELFKSNPSQAMIEFIQGLKDSEKHGISAIKVLDDMGITEVRLRDSLLRAANASDVFEGAVKRGNEAFNENTALAEEAGKRYGTTESQLKILRGQLNDVAITFGGPLVAALNSAISAAKPMIEALANMAEAFASADPKTQEFILKMAALAASAGPVLKVFGKMTSVFGKTISTMFEKAGNIDSKWKQFIVTPIKNGSSSALQAVKGFVSKYKSNLAGLESAGINVNLLTRFTTLKDTIVGLFPTLDTFGANLRASQRQLNMLGEGNKVTNFFRSFSASLQLSNSKLAKFASVVINPIGSLRNLSSAAGKSGTVLSGLGVAASKAGGGFRTFAATGIRSIASLTGAMLSNPITAILVAITTTIVGVVQAWKSNFMNIQGYVKTAFSGIVKSFKSVLPSSASVTKTIKGLGNIFKWLGTGTLVGVTFAIAGFVDGLRAIITVGKTAVNAIMAIANGVKGLWQRLKGDSKGADKSFKDVKKSLADIGKDWDTMFSDSALKKAAKSTEELGKKSKDTTKAMSMNMEEVSNSVENYSSKLDEAKQAMTELFSQQNGSTAGVEAYFNHTLDLVTNLKEQQKKAVETYNKQIEAAEGKSEAEKQKIFANASTEYMKAVQSNNSDLLKVYTDYSNQLKNNKTVEGQELTDQQRATLQNQTNIIRDQLLDQQKQFVEAGVNKLNNNQALSEQEKEQTLSSLKTFGEIQAQQVQENNAQIQQLETQKNQAKTESEKAAFQNQITQLQTQNDQIRQSELEQGAQLLAIISQNGANKIAVTADNLAQLKGVTDQQLLGIYQSYVNNGASIDQQMALLAGMLRQRGIDGSNGLVQGLQSNDPKLWANMSKADIVNTLQSLPPDLFKNGQDGKNKLIDGLNSGKVEINNVGQELMNQMNSGVKNKKAEAEKTSGDVASSGAKGAKSKGKEYNSGGNSNAGEYNTGLAKQKSNAKQKGAELGSAPVEGVKTKASAMRSVGEQLGRSFVQGLASQVGSANNAGRELGNAVKSGAGSVNMTSVGSNMAKGVASGIRASQGEAVSAMQNLVAAVNAEAQKKAKIKSPSRLLKYDVGVFLAQGVAAGIREDTSVAVQSAKDMISSIHQSITGSRLIKRSNAIEVKHSIDNTPMGKMVEILEEIRHLTVVMDTGQVVGALGSPMNLNLAEQQKQDGRYRS

SEQ ID NO: 2 - DNA, 39290 bp, Enterococcus hirae
atgagtaaaacaactaaaaatccactcgtcaaaccttttgtaaaatgggcaggtggaaaaaggcagctaatgcctgaaattattaaatataagccaaaaaactataaaaaatttattgaacctttcgttggcggtggttcagtgtttatggaacttcaaaataataacactgtaattaatgattttaattttgaattaattaacacatatattgtaattagagataatttagatgagttaatattggaattggaaaaacataaagagaatgattcaaaagattatttttataaattaagagaatgggatagaaatggaactttagaagaaaagtcaaatgtagaaagagcttctcgctttatatatttgaataaaacttgcttcaatggtttgtttagagttaattcgcaaaatcaatttaatgttccatatggacattacaaaaatcctaatatagtaaataaagaagttttgattgctgatagtaaatttttaaataaatcgggaattaaaattatgaatgaagactttgaaaaagctgcaaaaactgctagaaaaggagattttgtgtactttgaccctccatacgcaccactagttgaagactcacaaagttttgtggggtatactttaaatgggtttgattatgaagaacaagtacgattaagaaacttgtttattgaattagataaaaaaggttgttttgtaatgttgtcaaattcatccagcaaaattatacatgatttgtattctgactataaagatactaccgttataatagaagcaagtagaaacataaattcaaaggcaagtggtagaggtaaagtggatgaagttctcataacaaattacaattacaggcaaagctaacgtgtaaggaagtggtaatagtgaaaaaaggtaaaaatgatgaagcttgggagaagctgtttgataaatatgatatcttaaataaaatcgataaaaatgaaacatttagcataagttctaaacaaatcaatgagttccgagaagccagactaatgacaaaattcgatcattccaatcaattgcctgaaatactttcaaaaaataatattactattcttcctgattctagaggtaattatattcttgggaaattcaaaatatttgaagagttgaaacataaaaatctcaaaccaatttctatgcaaatacctgattttatacaatctttagatattacaaaaataacaagtgaaagttctgcattaaatattgcccatatgagtcaaatgatagattcggtaatgcaaactaaacacaatgaacctcggtcattacttactttaagtggaagaatgtcaagtggttctctccagtacaatatactcaatgttgataagaaaattcataaattttcagttgaaaatgcacaaattgaaattgatggttcttatgaaaatttgaacaatatacttattgtcgaagctaaaaataaaattcctttagactttaatatcagacagctatattatccttttcgcttgtatcaaagtttaaatactacaaaaaatattactccagtcttctttacctatgccgacgatatattttcttttcatgtatttaaatttacagatattatgaactattctagtattaaaaaagttgaacaaattaattttatcttgaatgattccttggatttaaacttagaagaagtaaaaaaaattagtgcaacagctaaagaagtcgaagaaccaaaaaatgttccatttcctcaagcagacacttttactagaatacttgatatgattgattatatatacgaaagaaaaaacaaatatgaattagcagaagcatatgattttgatttaagacaaagtgactattatgcgaatgcattagtatatttagggcttgcaacaaagcagaaccattatttcaagttaaatgatgaaggaataaaaattaaaaatatgcacaactcgaataagagaaatgctttgcttatctctaaaatattatcgcataagccttttaaaattgcatttgattccacactaaaaaatggtggcaattatgataggaaatatatttctaaaatcttactgaataatgtggtgtcgataaacagtgaatctacagctaatagaagaatgcagactgttgttgcatggttaaattggatatttagtgtaatagaataacatttaatcattttttagttagattattctagctcttttattacagaaaaatagattatgtaccctgtaggactcgaacctacgaccggacggttatgagccgtctgctctgaccaactgagctaagggtacaggttgttgccactttgttcatacgaattatccattaaagaaagggttgtggcaacaaacctattatcgcataattttggagtgtgactagtaatgatagtgaacatatgcgataataaatatattttaccgaacattttttagaattgtcaatacgattatgtacagctcctcaacgaggagctttttatttataaagttaaataaatatccttaatccgaacatcattcactgcaccttcaccatttgcttgattacaacgacggaaaatgacatcgattttcgtgccttttttcacccaacctagatccactgtgacgtccatacctagagcatcaccacctttgtatccatatgctttcttcacgtcagagcgtttaatcccttgtgaagctatacgagtgatttcctttgtggtgccatgttccatgatcaagacttccgcatacttaccaattggaccatctggtttatctggtactagccaaccagcaatattcacctttttatttccaacaaatttgaatcgttccaacttaccatatgcatttccctgatggactactttacttgctgctactgctttgtcatgagcagacggtgtttgtggttttggttgctgtacttgtaccgattctactttcacttgattacttgaagtttgacacttacctgatgtggcatatgctttccaagtattttgatcaccataaaacttattttggtcatatggtgtcgaagtatactgccacataaccgcatttgtccaatgtttcaaagctggaaattggaattgataagctgctacccatagaccataatcagctttaacaatcgctgagaaatcttcttcaaataaaacagaagcggacgtatacactaacgctttgatacctgttttttgttggatacgatctaacatttgttttaaaacgcctgttccttgacgtccatacatttcataatctaaaacgagaattcctttaccaatgtaaccttgaacattattaataaagaaatccgtttgtgcttgccaatttgaaccgtcaataaaatgatacacgccaaagggttttccagacttgatagcttgttgaacaaacggatcgcaatagcgatcaacaaaattacacccttccgttgctttaaacatataagcatctgcgggataatctttaatactttttgaaccgttattattcgataaatctactactttcaatgtcatttttcatcttctccttcatctaattctttgattccatggttggttcgtttccataactgatcgccatacactgtaattcccaccgctacaatggctacaaaaaagttaaatacagtatacccaccaaataatagtggtgtaccaatacaactaataaccgtaagtgccaaaggaattccccagttagggaacttaggaatttcctttaacacttttcctgctacatatagtccacacattgcaaggatcatttcagttgagagtgattccatccatcttcacctcttttcagagcataaaaaagaagcacaaaatcactttcgtacttctttttcaatctcatttactttgttttcaattcgtttcatatcagagctcatattcataaacccattttttaactcattcaacgtggctaaaaaatctcttcgatcttgttttgaactatttctctcatcttgtaattctttccgataggaaaggatcatccgccatgcagcaaaaatgataatccctactagaataatggttaatggtaaaaaaataagcccgtctattgcgactaacttagaaaatacttgatcaatgcctttcatatcttcccacctgctttctattcagtgagaatctctttcgcttcttcttttgtaatacttccttgtgcaacatagctcatgacgtccgcttttgtatacacacctaaatcataaaaaaactgaatatcttctttacttggatacatttggcacgcctccttctgtaattactgcctcatttggaaatacaacatcttgaattctttccaccatttttttcagttttgttaattctttcatggtattcgctgctacctgattggagcgaacatactgatcataaggaactcctttcacccaaatccactgattgttttcccaatcaaaacctgcaatcatcacatctggtcctttaggtggttctacttctgtaaatggtcgtgaagtcgttgattcttttggtgcaaaccagacttcataactttgtccgactactttataaacaactttcatattttcattcataaatcttcctcctaatgtttaaatacttcattccataattgttgaatttgtgtttgcattcgatcaatggtagggtctctcttgtaataaagcagatctgtcaaataaattcgataagtaaactgcaacgtagtttttccatagtataaagaagtatatgcccctttttcacccatcatgagaatattcactcgtccttgtgaatctaagaattgttcacttccattttttacaaccgaagcggacattgtttgaaatcttttttctggatttcgttgatattctctccattgttctaaataattgtcataccataaacaacccattcctccttgtccgttactccaactatcagctaccgttccatgataaccatacccataggtacttggagtgatcgaaactatccctttttcagtcaattgaacttgttgttctaagatatttatacctaatgcttcatagtaatcttctcctaaccatcgtttgatttcctccactacattccattggatgcgtaaataaggatagttaggattattatcggaaccagatgaactagaattatatgttctagttccacgtagagcttcataaccaattgcattgactgcacttggataagcattaacttcaggataacgcgtgtaaggagtaggcatttcaaacctgttttcagaaagaaaattgacttgactagcaatattgggattttcagccatactaccgaccacttttcctttaaaatcaagtgaccgtgatacctcgaaataaccttttgtaaatgcctcaatcaattcttttttcgtgaataattcattttcatcaatgagttgcaataatcgattggtttcgctttgattaacttctactttttgactaagtgattggacttgttcggtcacttgaccaacgctagcctctaattctggtcttagtgtttcaatggcttctttttcactttctgctaaatcaaaaatttcttttttgatttgttcgaagtctttgatgtatacctcacttgcttcttcaatttcactttcaatttttgaacggataactgtaaaagtgaaggctagctcatcactgtgagagccatcttcgaaatcaagatacacgtatccttttacttcgccttcataatttaataactggtcaggcagaggataagtcacaatcccactttcagggtattcaataatcggttgactatcgattgcagtaaatttcttttcttggccatcttgattgatggttagtaagattttaaatgtagtattggtgagatcgacaatttgataatcttgatcacggaacaaaaattctaatactacagaacctttgtcataactataaaaaacaaagcctgtatcttggccatgtcttccctttacttttgtattgacttttattcgaccaatttttttaaacgtcatttactacacctccttcccaaataataaaagctattctactcagtcgcatcttgagctagaatagcttgaactttcttttttagtgtttttggcacatcatcaatcgttttctttccttttctgattaagtccgcatagatgttttccatgttactcactccctaatgaagattcataaatttcggtcattgctacttgtaaatctgtcacttgattattcaaggcttcgttactctctttgaaagcttgattttcttcttgaactttttcaagttgttgttcagttttacgatggatttcttctaacaactccaattttttagagaaatcttgtgtgactacttcttcccattttcgctcccttggattccaaaattggcgatctaatggaatatctggtaatggtggtacagaagtatacggcactccttctgggaaatcatctggcatgttttcccagaccttaccccctactggataaagatattcatacattgttttcatcatttattccccctattgatttggccacgcatcatttgtaaaatagctgacggttccagaacactcttgattttctggtaaatttgtagtagaaaccatcacagcaattcccgaagcatttgcgtaaacagataatgcaagatttcgattggttttattcgccaaagttccaccccaatcctttagcgaagttggagtatatccttttggaaaaggcattaaaactttccagccaccaaaatttgctgatttatttgtgatcgaaaaattggctactacacttcgtccatctcgttcaaatctgactgaactttcattggtgaaatctgttgtattcgtcgtttttactgtttttgaaacaaaacgatctacagctactggtacatcattcactgttggtgtttgttgaaaatctttgaaaccaccaatgcgttgattactagaagtatccacagcttccttaaaattttggttaatagtttctgcaccattctccatacctctataaatttcttgaaatggcattaaaatccctcctatatcgataaatcaaaaacgattgatcgattattttcttcatcaataataagatatttattatcattaattttattcggtaaataggttgttttatagtccttcggtattgtaactacacatttattggaactaatttgcttaacactacaaggaactgttatagaagcgctccctccaaagaaaccttcgggttcagtccctaatggaactacaccaatcccatatgtccaagttctaaccacaattaacggattcgctcctaaattatgctcaatcgttacatcgaatccatctggaatagaagacgacaaaatcttttcaatatattctaatctttcgtccagagttgcaaaatttccatacttttcactgcttctagcattaattaactcgctatctacagtagcattagcaatcacacttttgaaattttcttcaatagtagtttgtcgcttttcaatctctgactgacgtttctcggtattttctgttaaaagtttaattttattgaacaatacactggtatattccatcattcttgctagtgattctcttacatgtcgacgatacattttagttcttatccatgtagcaaatgttcttgaaataggatcaataatcccatactttatttcatcttgaacctcatcaacatctgttggatctcggtaatctacagacgtattaggttcattcgttggttgtgtatctttaaattcttgtgtcaacaaaattcacctcacttattttctaaattctcaactcgtttgattaaactagaaatagtctcatcagactcttctcgagatttttttaaatcagttatttcggagcttaaattagtttcaacttgagctataccatcttttagggaattaatagattctgaaagtttttgagttccttcacttaaatttattatttcgttattttgctgagacacttcattttttaaagattcctgtttttttattaaatctgaaattgactgtgttccagccgaagcatttgctttgatattaactaaattagattgaattgtttttatttcattctggtaatctgttaattttttctttttagaacctattgtaagtgttactttttgaggtgctaaaatactaaacttcttttcaattacttgtagcctttctaccgcatagagaaattgattatctactttgtaactgtttcctaaagtgattaattcataccgtttatccaatagccctaactcaatggcttcaactgtccaagttaccaacatcaagctttggtcttttagccattgcaaccctcgacgttttaaaattgatgggtctttgacatttgaaaattctacaatgcccgtgtttaatccaaattttttgattaacgcttcatcatcaagataattcttaccgccatttactttttcgatggtatatttaggtcgtgaaaaatctgtccccacttcaatatcagtatttgacgtatcttcaatatcttgaccgacgggcacaatccttgtaaacaattcagaaatatcaatatctcgagtagcactttttagatttttggttaactgtaaaggagtttcactgttcacaccataattagatagataatctaaataatttatattcccaacgcgtcgaagtgttaacgtaccgcctagcctatccaataatttttctttgatggtatcagctgtgctttgatagcccagccctctcaatagatcaccgttatctataacgtcaacgttacctaacttaaaccttttatagggttccacttgcttgttatgaatatcaattattttctgcaaataatctctgacgggcattcgagtcggcttcatatatgtttgcacagaatcatataaaaaagctttctcatcttctataagaaaagattgagaaaagctacccgatgtatccattgtgtttgttattttagctactcgaccataaaaaatttcttgttctcgtacagcatctataatttgaataaagttaataataggctctatcttttgatagtatttattgttaatgttgaatgtgaattcaaacgtagaaattcctaatccgtttaaagatagataaacttcactctccttaattttttcaccgtagctataaggctcgtgaacaattttgggatttagacgattcggattgtcatatagtaatacacgatacattaaaccatcacctcactagacataaagaaagagatatgaccttcgccaaaaatggttaaatgattgattccttttttcagtttaaagaagtaatcttgtgattctccttttggaacctttattgttgttccgtcatctgtagttaatttcattgaagacgttgcctttatcgttggactagaagcatttgctcccatattgataaggaaaatttccctttttctatgaatatagtagcctgtccagttatctacactatcgtctgtgaaaaagtcctcgtcaaaaatatctgaataagaaatattttcccttaaagcaaaagggtaaacatcaaattctacagttaacgttaatgagttacttgacgcatcatcttccgctttcacacttttacattttccataccacctaagacctgaacgcaaccaagagtcttcaatataatcaatcccttgtaacattagttcttctttcacttgggcttccaacgccttacgttcatcataaggcgtattagatcgccaaaaagtaactgtgacaattcgattactgaaaattcgttcaccagtcaacattgagaaatcatattgcccttgcataaaaggaatttgctcaataatttctacttcttccgcagaaggagcatcgtgttcaataatgtagaaaccatgttctttgctgttaaaacgaccttttgccatatattctacaatttcaatcaactacgatacctcccatcttgcttttgttgttctgctaaattaagattcatcgggctacctagtgctcccactacttggccagtatccatcacaacagttaaatgacgtatttcttctaagatttctaccattttccccatcggcgtattatctatagaatgttttacctcaattgcatttgatcgttttatcaaacgactgcctgtaatagactggtgaatgcttgaaatcatatcttttgcactttgtacggcaactgacgtatcttctcgaatacctgctgccacaccctgtgcaaggaaaacaccaacgtcatatttcaataggcgtgatggagatttaatctttgcttttttctgtgcttctgcattaactgcagctactaaattttgcatagcagatactgcttctccttggctagctctaataccagaagcaacacctttagccatattagatccaacggatgtcatattgactgaaccagcaccactttttactgcgtttcctaattctctaccagcgttattagctgaaccaacctgtgatgccaatccttgaacgaaactacgcccaagctgttctcctacgcttcgcatagcagaagctttcgtttttactccttcaacaggcgctgatcctaattctgcacctttttgttttgcgttgcttttctgtttcgctagccctgtgttatactctccagcattagaattaccgccgctattgtattctttacctttactttttgcgccctttgcaccagatgaagctacatcaccagaagttttttccgcttctgctttcttattttttacgcctgagttcatctgattcattaactcttgaccgacattattgatttcaacttttcctgagttcaacccgtcgattaatttgtttttaccatcttgaccgtttttaaacaaatcaggcggtaatgattgcaaggtattcacaatgtcagcttttgacatattcgcccataatttaggatcgttgctttgcaatccttgaactagtccgttagaaccatcaattcctcgttgacgtaacattccagctaataaagccatttgttggtcaatgctagcaccgttgtttacatacgattgataaattcctaataactgttggtctgtcactccttttaattgagctaaattatcagccgtcaccgcaattttatttgcaccattttgtgaaataatcgctagaagctgcgctccttgttctaattcactttgacgtatctgatcgttctgtgtttgtaattgcgtaatttggttttggaaagccgccttttctgattcagttttcgcttggttcttttgtgtttccaattgctgaatttgtgcattattctcctgcacttgctgtgcttgaatttctccaaaagtttttaaacttgataaagtttgttctttttcttgttcacttaacgcttggttgttattcagcttattcacaccagcttcgacaaactgtttctgttgatccaacaattgatcacgaataatattcgtttgattttgcaaagttgctctttgctgatcggttaactcttgaccttctaccgttttattattcttcaactgattagagtaatctgtgtatactttcaacagatcgctattgtttgattgaacagccttcatatactcagttgaagcattggcaaaaatcttttgtttttcagcttccgatttaccttctgccgcttcaatctgcttattataggtttcaacagcctttttctgttgttcttttagatttgtcactaaatcaagtgtatgattgaaataagcttctacgccagccgtgctaccgttttgctgtgagaaaagttcagtcattgcctgtttagcttcatcaagttttgatgagtaattttcaacactatttgatacctcttccatattcatggacatggctttcgtagtgtctttcgatttcttccctaattcttctgtgcttttagctgctttttttagagcagaatcagaaaacatggtatcccagtcttttccgatatcagctaaacttttcttcacatctttaaatgatttatcggctccttttgaatcgccttttaatctttgccaaagtccttttactccgttagcaatggccattattgcatttactgctgtctttcctacagtaataatggctcgcaatccatctacaaaacctgcaatagcaaaagtaactccgacaagagttcctgttcctaaccatttaaaaatatttcctaatccttttattgttttagtaacactcgcggagctaggaagtacacttttaaacgattttactattccgctaaaagcggttttcacgtagccttgaatgttcataaaattggatttccaagcttgcactacaccaactattgtagtggttattgctactaaaattgcagttataggattgctcaacatagctcctgttaaactagctatagatcgtatacccgttgctgcaaatgttctaaaacctccacctgcttttgaggcggctacaccaagtcctgataaaaccgtccctgatttaccagctgcagaagataaattccttagcgacccaataggattaataacaacggaggcgaatttcgctaatttgctattagataattgtaaagaagcagaaaaagaacggaaaaagttagtaactttattcccttcccctagcatatttagctgtctttggcttgctcgaagatttgctccaaaagtgtccaatgtgggaaagagacctacaatggtatcttttagcgtagtaaaacgggtaagcagatttacatttatccccgcactttcaagccctgcaagatttgatttatatttagaaacaaacccttttacagcttgtaatgcgctactagaaccgtttttgataggagtaacgataaattgtttccacttgctatctatgtttccagctttctcaaacattgttgaaattgttttgccaaaaacactagtcattttcccaaacacttttaatacaggaccagcagaagcagctaatgcagccatttttaaaataaattcttgagtttttggatcagctgatgcaaaagcctcggccatatttgctaaagcttcaatcataggcttagcagcacttattgcgctatttaatgcggctactaatggaccgccaaacgtaattgctacatcgtttaattgaccacgtaaaatctttaactgtgattctgtagttccgtatcgtttgccagcttcttctgctagagctgtattttcgttaaacgcttcgttacctcgttttacagcaccttcaaagacatcactcgcattagccgcacgtagtaaactatcacgtaatcgaacttcggtaatccccatatcatcaagtactttaatagctgagattccatgcttttctgagtctttcaaaccttgaataaactcaatcatagcttgagaaggattactcttgaataattccgcgaactcttcgccagttcgaccagtaacatttgcaaaatcttccaaacttccagacgccttgcttgcttctttatataattttttcaattctgaagctggtactcccatttgtttagaaacagctgttaattctttaccaccccaattaacagcatgaacaaatttttcccaagacactccttgtatagctacagcttgttttaaaggttcaaaagctttaacccctgtttcggtggctaattgcatttgtaccatcaacctagaaaaagctgaaccacccgcttcggcctctataccaacagatgataacgccgctgcaaaaccgacaatgtctccttcagtcataccaatttgttttcctgcaccagccaaacggagtcccatttctgtgatttctgattcagtagttgctaagttattccctaagtcaacaatagctgagccaagattgctaaatttatcttgagacatttgagtaatattagcaaaacgagctaaggaagtagcagctgtatctgcagacatatttgttgattcgcccatatcgatcattgttttagtaaatccgacaactttatcagtttttattcctaactgtccagctgcttctgctacttttgcaatttcttcatgactagtaggtaattcttttgctaaatctctaaggcctttttctaaatcatcataagaataaatgactttaccgttagaatcgaccatctcatcgttggtctttttaacaccagtaaatgcactttcccattttacggctgcagttgtgactgctccaacagcacccgcaattgggagtgtgatacctttagtcatcgaaccgccgactttttcaatgctttggccgatacttgcagttttatcaccaaaacttttcatcgcaccactaactgtgttcaaattactgggaatatcagaagcattcgaactaagtttttttagcgaagaggtagcactccccattgtctgagtaaaccctttatctattgctgtaagtaccgctttgactgttttactttgtgccacgttgtttcctcctttcctcaacaatttttcttgcttgttctaatcgacgagcgttttcttctagctcacttagcttttccgcttctcgttgcgaaatttcccctcgcacatcgcgttcaagcttttcaaagtcgtagacgtctttcacttcgttaaaaatatagcgttgtcctttttcgtctggcgttgtaaaaatacgtgtagctaacgcgttaacgtatagtttcctttcttcgttaattgcacgtaaatttacagcttttatccgtaaattaaattcataaggggtcatacgctcaatttcttttaaagtgatattggggaaatgttgaaaacaagtgacaactatttcgtcataatctaggctgtcgtttcttgttgattggcttgcatctgttccatgtaagccatgattttttggatcgcttctagtgcttttttcgttcgaagagccgttaacggtgcttgctccaagaaagagataaaattttcaaacaacgttaaagcctcatctgacgtttctaagtagtcgtcaatttctttcgttgttaagtcatcgtaagtaattaacgctgcgtgcattaatttttgaaaggcaaaagcgtcgccatcttgtaactctccgatcagttgaacgaagccgtccaattcttcaacgtcaggttttaatgcgttaatttcgtttaaaaatttaaaaccgaaaaccaaaggatatttttttccattaattgttgcgactggttttacgtttgttgacatgtaaaattcctcctaaaaaagcgacaatgctttcacattgtcgcttacttcttgatttttaattatggtactaatgctaataaatctgttttcgttgtttttcctgtaaaatcaataccgtgagcagttaaccattctttgatttcaggaatagtatttgcttctgttggtttattttccaaagagcgccctgccaatacagtaaaagctggaatagctactttttcagattctttttcatcttgcacacgtacaagatgatacgttcctgctgttacttttgctcctgcatcaagtcctgtgatagttaatggacttgctccttcaaccactttttcactacctttataaatacgataagtaattgccatgattattcttcctccttcacttttacaacggcaccatctgctgttggcgttacactttcaattttaggtacctcaattgttttaggtgcgtatttttctactggctcttctggttctgctccagccaccgtatcatagaagaaagcgcgtgccagttcttcattttcagtatcaactgttgcccaaccttctactaaatcaccatttagcaccaatgttggtttgatacttgaattagaatcagattcagcagaatctccgaatgaatccaataatcctgtaccaaattcagcttcgtatttccctgtttttggatcttttttatcaaaattaatgcgccatacatcaatttctaacccattacgatacgcatatttcaacatgttataagtttctgttcctgttcgtaaaaattccatttcaatagaagctgatggcattcctgatgtaggaacatttccgtcttttgttgattgggtatctgtttttgtttctgacttatattcgtgtgaaatttctaaagctagcaactttgctgctgttgttgcacgttcacgggttagctgaaacattaatttaatttttttaccttgaattgctttttccatttcgagtttccttctttcttattcaaattctaacgtgatgtcaagtacaccgtgtgcaaggctcgtaccaaaattggttgtattttcataaataacttctgtgctactttctatcactaaccaattaaagttcttagtctgatgcaattcatgaacgatttttcgcacatcggctaatgtttgatttaattctcgacgtttgtcgtcatgattataaacatgaatcataatatttgttgaacctaacgttcttgtttttgtttgtctatccttagaccattgttcacctaagaaaacaaacggataagaagcctcatcatctggcaaatgcgcataggtttcataacctgcttgctccagtgtgacaaataatgcttcataaaattcagaatatggatctttaaaggtcattttactaactcctccatatcgttaaggaatctcttaatagctgccgcatgcccttttttcatatagaaacgtccatacatgtaacgcgttccatactctacatacgctgaataatcagcaaaagctctcacttctccagtcattccatcatctttaataaaagatacttctgttcttttcaagtaaccacttttaactggtgtttcttctgcaattcgatttgccatataggcagtatcattctttacgattgcttttacatcatccagctttttcgcttcttcaatcgcttcgattaaatcgtccaaccctgaaatttctacgcgataagtcatcgatactcacttccatacactgttgtgcctttactaacacgcaaatttttcacaacagtaaattttcgatttttttgttcttcttcatcgtagtattcaagaaagcctgaacgaatagttaggcgatctctaaaacgaaaaatgaccatttgctcctttacagtaggaaaaatggtcatttgtttttctgttccaacttcggttacactgcctatcaagttttccgaaatcaattcatgttttttattgtaataattaatacaggttctcataaaaatgatacctttctttttctggttagtcctttttcttcaagataatcgttaatttcactttgaaattctccaaaatcgtctaaattataagaaatggtttcttctgactgggaatgttgttccattccttcaaaccccaaccgattatatcgtttaacaactacggcagacacgatataatctaattcatcgggaatctcgtcagctttaagttttataagcaactgtttttcagtcatttctataatttttctgattttttctttatctttattaaatgtttcttctgaaatatctaataaaaggcggaaatcattaaggttcattttttcacctactattctacttcaataactgccccatctgccgttggtgttacctttttaacggtcggggcgcttactttgaagtgtatgatacataaatcgctgggcgtgctttttcagttacgatagcatcgtaatagtttaatcctttgattgtatctctgtagccgtcacgatcttgtgaagctggaattagatcaatagagttgtatttttcaactggcgaacaaaccatcaaaggcacaagaatataattaattttcttcgtagaatctacctgcaaacgagattttgcaactttttgaataatagtatctgaaccgtccaactgcgcaactttacgattaatacccgaaatttgttgctcattcgtagtaaatgtttttgacacaccttttgcattttttaatgctgaataatagtcagtagatgcaaacatgataaacggaccgacaatttctgcatccgtcatgtaggcttctgccgcatcataggaagctagagaattttctgtggtaatagtttcttctactgttttccctacatattttccttcagtgtcgtcttcagcggcttcagcgaatgccgcttctaataatcgttgtacagcagttcgatctttttcaggaatcgcaattaaacgagtatgctcttctacaagcgcttgaacttcgtaggaagcattttctgattgatctaatgtgtctaagtcataaccaaaccaacgctctttctccaatttgaacgtttcttttgctacatcaattttagaacgaccattagcttcattacgtttataatcactagcagtaaaacctttcatcttattgatgcggacttctttcgctcctacaaaatctgcctcagttactgcagcagctccaccttttaataagtcccatacttgagaacctgtggcaaattctttgtcaattgcttttaaatctttgctatctaaaataattggcataatttttcatctcctatttcttttctaaatttttagctaaattactgcgccaatcagtctcttttgttgccgttgcaatatttactacttgacctttcagcaattctttttggataccctctcttgcttttgaaatgatttgctttaattcatctacagctttttttgtatcctcatccgtatcttttataagcaataaatctgcttgggatgcacttacataatcagaaagaccgttctcagataaatcattacggacagactcggcacgatctaaacgatcaatgcgagcttgtgcttccttttctctcttttctgcttgagcttctttatcagctgcttcttgttcctttgctttcacacgttcttctgcagtcatttgctcgtaagatttttgcttctcccaatcagattttgcttgttccacagcctttttagtttctgctgcaaccatcttggcaacatcatcacgagtaaaggttttccctgtctcttttccgtctggatttttatcttttggattctgagaatcatttgtcgatgaagttccagatccgtttggattgtcagactttggatcatcgggatttggatcatccgcaaaaaattgtaaattcatcggtaacaataaacgtttattagctttcattttgattcctccagtcattacgtgaccaatcgaaattaataggttacgcctatcaatcgaaacagctttctctttaacgcctgtaagcagtaagaaggcaataaaaaaaagactaacgtttgttagacttttcatctttatatgctggtgcagtgctacaccgacaccaattatgaatagggcttgcattgctacctggactcatttctgaaactttatgtggatttgcgcttgctatccccacacaaataggacaagcgcttggctctacgattaaattgtattcatcatatccgtacttttcgtaactttgcttttgtatctcactttgaattctagaagactcactgatcattaaccttctagccacataatcagccgtttcttttcctctcaaactatcaattactactaatttgcgtaattctctagctagaatatcagggtgtttgcctgcaattaaaccaactgtaagcaatcgatcaatattagcttttaaaatatcttgattcaaccacaaacgctgtgaaaatgtcgcattatgaaatgatccatcaataattgctctagcaaattttcgatagacctcttcagaaagtattgactcacctaaaattcctgcttgtcgtttgaattcttcgattgcttcgttcatcaactgattattgaaataagtttgtagctggtccgtattatcggttaaatagataccaatacttgatttcaacaattctaagcgatttatcttcattgttaagttatataaccgtagctgatcgtttgcttcttttgaaaaatctcttgtttgtacatagagttttactttattaacaaaagcctgaacttcgtgtttacttacacgccgttttgcttcttcaatagaaatcttttctcttccagcataatttgagtagaattgttgtatttccgactctatctttatccacaattgtttgtaacgtctgtggatttcctgttcataacttatatgtcgacttagcatttcttcaatgtgttttgcttctcgttcagtccaataattactcatgttcttcggtcacttcctccgtagtttgagtaatttccgtaaaatcaatttgaggatttaaccgatcttccgtttcttcatcctttatacgttccatttcttgggtcacatcaggaacaatcgataatacacctagttgcgtttctcttgagacaatcccttcaagtttttgtgcggtttctgcttcgtctttaatattacgcggaatgttaaactcaaaattatattctaaattaaaccattctctcgctttagctgcaggtacgtttgtaggtaatgaaaaaatcattttgtacatttgcgcatatccttttttaaacttccttgcttttgcttgtgcgaggtttctagggttttgcattttaaattctaacgagatacctgaggcattgttgctgaaactttcgtcatttgcgttgtaagtcattgacatttggtaaatcagacgttctaatcgatctaataaattttcttgagtagcgtcagaactaggtttgtctaaaaaattaatgtctacagtttcaccttcgtttaaaggatctgcgctgttaattactcgattatcacgcaaaaaggcagcaacattcttatcagttaaatctacaccgatcatttttaagtaagcatctgcaaagtaactcacatcatttgccttttcagataatgcttcgttgtaattgttaatcagagaccacaccgattcgatacgcccttgtcgttcgtcattttccataaactcaatcataggcacttctccatatggattagtgattgcctcttttccgcctagtaaataggacaaagctttctgaaaaacagttagcccttgtttaggctccaatcgtttagaagtcttggtttgtgtaaaaataaacgtctcagtgctattttgaggataaactgttgctgttagttcatctcttgtcattttgttatataaaactgcaaacataggtgcttttaataaatcatctgcgtaaacgataaacccttgtgtaggttttaaataggtcacacacgtttcggcttcttcattttgatataaaagcttataagcgtgcccataaatagcagttagcttagaaagctctgcatcgttgtcttcttcctcgtttcttttacgaaaatcttggacaaattcttttatctcttcatctggatgagtaatctttgttggcttaccgttaaagaaagctgcagaactatctacaacatagcgagcaaaatttacagctatacgatgatctggttttccaattcctttatttttttgataataaatgtcatgttggccattgtagagcttctctagctcttcgtaaaacccgattagttttcgatgtttattaatatatttgtctactaactgttcattaatctctgcatttttatcacaataaaatacacgatttcccaaaaggtcaacgaactctcgtattttactttcagtgtttgttctacttacttcatccgtcatcaaataacccccttcacactttgtaatttaatcccacgtgttttcttactacgatgttctactgcatatcgtaaggcatctatcacgtgattatagctatcaataggctcattggtgtattcccctgttttcttatctttagcccacgtatagttttccaattcctcaatcagtttgacacagcgatcatctactattagctcgtactgcaataaaaaagaaagcccctgacgtatcgaatcaggacctttcttagctgcacgtattctagtaattccgttcttcttgatttctgcaatagatttcttttctgctgagtcagcagtaataatttcttttgaatagcctaaatctttaataactgttgcaatctcatcgttcaacattccttttttaacatactcttcaagaacatatatttctttgttcttctcgtctactttaacgtgaataaaagcagatggatcatttacatacccaaagtctaggccgaaatccgaatcaagctgccttagcttttcatcgtgcttgtccaatctttttctttggtaagttggaaacacaagcttatctagcgtagcaaattctcctaaagcgtatatgcgataatacgctgggtttcgcttagctaaatcctcaattacctttttattttcactatcaagaaaccgattgtctttatatgtgctgtgataaatccctgttctttgttgatcgacttctgcttcctcaccaaagaaagatttatatacccaatttagtttagaaactgggttaaacattaaaaagatttgacgtttcacatgcctacgctcacgtaaacgtaaagtaagttgtgtataatcttctagcgtaaattctgttgcttcttccatcactacatcagacagacctttgatagattttattttctctgggtcgtccattcccttgaaaaggaactccgccccatttggtaaagtaatcctaaaatcggtgttgtttactttacacttgtctagcagtccccaatccgaaagacacgctttcacatcctcgaaaatagagtcttttaagctacgccctacttttcttgtaaataaaatctttcttggtttcttccacttctgacaggctttaaaaacaaccttttgaacaactccgtgactcttgccagatgaagcgccgccccaataaacctcagtaaatttagaatagtcaactaatcgatcataaaatgatttgttaaaaactcttgacgggaaattaaactctaaaataatgttacgtttcttcgtctgcatcccattcaccaaccttaattacaatatctcctgtttgtaaatcgactttatcagtgaacagtgcatgacgtttaccaagaagttctgcagcttttaatcgatcttttgcacccacatcaatatctacgattgtttgttcgccttctcctaaaccgattatcgtttcttctttgtactcaccacgcataacagccgttaaatactccaaaacttcttgagcatcggctgttcgttcgtttttcatttctgcaaggcgtttgtctatataagatttaattgtagtattttgtagtaatttagaagcatttgtgtttgcgtattttgaactataacccgctttaattgctgcctgtgtagcatttcctgtctcaatgtagaagtcgcaaaatcgtttctgtttctcggtcatcctcataatattcacctcctcaaaataaaaagaccactcaatgagtgatctaatatgtactacaggacccactatccttcgagggaatgtggattacagaaacatcagcgcgctatagtttccaacctgtatattcggttttactgacaggcagttatggattaccgtaaaccaaagtcactggcaaggaatcgaacctggcatggtcaaatcataaaacgttaaggctatccctcgacgtattgaccttatttttaagcgtctaccctttccgccacagtgacataaaaaaacggaatacctactatacaataattttataatagatatccccgtacgaaacagtattcattgctataattcatttatcagcgatggaagcgctgaaataactattagcgaggtatactttatgcacaaaacaggatcaaaaccaggcaaaggcgagtactattgcctaaattgcggacaaaacgtcacacttgaccaatctactgacaaattaccaccatgtccacgatgtaccaacacaacctttagaaaaggatagccagtgaagaggtcgatgttcgacctcttttaaattgcaatttctcttttgaaaaaacaataaggttttccgaaaagattaatttgaaaccatgccactgcttttcgctcattgttttcgtttctgtactttgtaataaaatgatgcataattgaatcctcccacttatttattttttagtaatttgctactgatttcccacgatatgtgtttccgtcactatcttgaggagcagtcccatctgcttctctatttttttgtacagctgatctatacttttctactgagtaacactcaattactctctctaaatgattttgataaacttttagagtctctttcaaatgcttgttttcttctagcaaaaattgattttctttttttaaatccatattaatctctccatttatataataaacagacagcaaccagttgatatagataaacaatggaaagtaaaggaggttttcacttccttttgttatttttttgtttagttgctgcctatcgaagctcaataaaacgatgagggagatttcctcccttacattttattttgtcgaattcctgtttcctaatctttcgacactatcataatatcacgttaaatcgtataatttgtgccaaatctacgccaaaaaggccaaaattgcgccaaaaacgccatttacgccaaaattatcgataagcaactactccgaaaacatctgcaaattctagtaaagcttctgatttcattcgattaaatgttcgagtagctacacccaaattatctgcaatttcatcatttgtcatagaatctcgtacacaatacgtatagtacagagtttgtctactaattaaacctagtctgcttagagcatattcaattgatttcaatttctcttttgattccatattctggataatggcatcctctaataaatttcctttacttggtgccttaggcatatcatcgataaatggagaacgaatatcaattggacttcgatctgcttttctttgtaagcttctatattgtcttaaaatagctcttgcattttctttggtttgttttatgtcagcttctttaatcattacaaatcactccaagatatgttataatgaaaaagaactttgttacaattcaccatactatgtagagacagccaattactggctgtctattttttataaaaatttttttattaattataattttttataaaaaataaaaatattaacatctgttatcatataaatgaacattgttttttatcttatatcatttaggaggaaactatgccatttatcgtttatttttttatgacatttgttattatttatattcctgtaccaacaattatttttttattttttagatttacagagcagcttactggaattgtaattatatataaattgcttcttttaattttattaatacttgatatcaagttaggatataacttattctataatcaaaaaattaaaaaacgaagttaccttctttttctctttctcaatacaatagaagaactaatgcacatttacttcttctttacgtatcataatgtttttctctttattttatgcattgcccaagtactcttattgaactgtgcttttttatttcctttatctaaaagttttcgcaaatttttattttaataaaaaatataatgaatttagacagctgaaaaatgactgtctattttttatgttctaaatatcaactccataagtggtcatccgtttaaactaatctgtgtaattgtcctttacttctaaaacatcatataagtctctacctcttactaactgttcattattttcattaatgataatcggtattaattccattttgttgctctcctttcttcaaatgctttgcattagccgttccattctgaacagccttttgttccaaacggcgttttttcttcttgatttttgattttgttttacccatttttatctcctaataactttgtagccatacaaataatttcgttaataaatagcgtaataacacctatacattgcaatctaaccctaccgtttctgtctaacattgtgactttcggaccgaacaacgtaataatgaacaatacccattctagtttcgtcatttcttattcccctcttgaataattactaacataacaataaaaagtacaataaatataaaaggataaatcattccgcttccccctcagcacaaaacgcatttcttataaatattacattcagttcttgtttttttatttttgctactctatgttttctgttattcattatgattcctccttatccaccccatcttgcgcaaagaattattcactacaaaacacatcagcaaagtattcgccattcttgtaaatattaagaaaatatttgtgactcggttctctatactcattgatattagctatttctgctacaaacacatcatcagtcttgctagctagattgaatctatcttttacttccattcttctatcacctcttccactgttccaccgatttgtatagcatccatttcggcttcttctttagaatcgtattttattcgttgagcaagcgcaccaggagcatcgtcaataatataagtcactttagtttcatcgaaaccagaaaaatatcctttgccaatttttacgcaatacaaagcatactccgaaaattttaagcattctgccgctgctttactaaaatttattccatactttgaaatagtaacttctggctctcttgcctgagaattcaatgcaatcaatttaaagtcttctgttagtttcataaaattaactccttgctactttttcatccaagcctgattaggtttagcttgtttcgtttttttctgtacaaatttcttagaatggttgttagcatttggattcttagaataatctttcacttctaccacttcaccattactcacataagcggctagttcagccatttcttttgtgttatatcgctttgcctttttcaaatcagggactccatatccttctgagtcgacataacacatcgcttttacaacgtatgtcacgctcaaacctccaatacctaatttctaaatgctctacgtattgtgtacgcttcgttaattattttcttcaatgtatccgacggatagattcgatggcttgctttcttggtatcttgttcatataaccaagcaagctgtgctagagtatcatcgtcaagagaaaatctcggtcttttcttaggtgtcccacctgtttgttttggctgtcccacctacacagtcgctccttctatttcttttgaataaagtgatacctctactcttggttgtttcgcatctactacgaaatgatgtgtgatttccacgatttcattccagccatcgtttggtaacgctcctgcattgactaaaccatcaagaataaacttaacggcaaacgcaatgttatcaggatctttccgtctatttttcatgtaccaagtaatcgacaagcacacaggtagctcgaaagataagccttgttgaatagcctctaacacggctcgtttacaccgattggtgtttttctgttttacttgatttcccttcatcggatgcgttcgttgaatattgataaattcgtttaaactcatcaattctccaggaatataaaacgtgttcatgcgattgctccttttactggttttaatcgtttatcggttgtttgagaaaagaccatcgtaaatccatcagaattgacaaacattcttgatgtcgtcctcgtaccgtaggcttctttcagttctttaccaagcaagttcgttgtgataatcgttggtaagttctgtcgtgcatccaagaacgaattcaatgtgtttacgccaaacgttcgactatctgatgcatcttttcctagctccgaaccaacatcatcaatgacaactaaatccgctgttttgatatctgcaatcaacgacccctcgatcgtttttctgagttcaggattgttgtacgaaaacttgatttgatccagcatttcctgtaatccgataaacaagattttcttgtcgtagtttgagcgcttcaaaacttcccaagccgctgccatcgctaggtgacttttacctgctccctgtttgccacttaaaacaaggtgacttggatttcctagcaagactgaattaacaaagcgtttggttacttcaactgcttgtcttgtttcttgatcgacaatttgataattctgtaatgtacaatcaaacaacgctttgtttggcacgacagaaccacctttgaaaaaattgatggctcttgctttcagactttcgttgtacattcgctctgtctgtaaatcttcctgaactcgcaatgctttataaccacactgcatacaggttggtttacagcgctctgagccatcggggttcttcgtacgccatccatacaaaggctgtccacattcaggacattcaccacgttggacaagcaccttctgtatcagcttttccatgatttctccaacggtttccatgtccacgcctcctctcaaataggcaactcatctgtgctaaatttctcgtattcaagcgttttggtttgttttgttttataatcacgattcgcttgcgctgccattgtgtcatatttttctcgcaattttttagcagataaaatattcgatgcccaaaacacattgtgctgactccattcaatcattccccgtacctggttttcggtccgcttgtcgatctcgatcattttccgaatgtcatctgcccaactttgcagattcggctttttgatttcctgattctgacaaatctgtttgaataactcctccgcgagaatgtaataaactgagtcggtgtcgtaaacacgctttttgcgtggttgcgacgatgatgttttattattcttttcattcttataattcttttcattcttgtttgtgtgcacttgttgttcacttgttgtgcgtttgatgttcatttgatgttcattgctttggtacaaagaccagttttgtattgatataacgctgtatttcgtagttgatttgatgttcaacattccgtttttttcaaattgctttagccatctccatacagaaccgctgttcacttgatgttcacgtttcacgccttcgttcatctcagatgtgatagcatcgcgccctgtgacgaattccccgctgttcacttgtatctcttttccattaaaaagtatcttgcgattctcatgactcgctttcatcaaacacaagctccataatttatacatataaggattggtccaaacgaatgaattcatcacttttcgatgtaatttgacatatcctgtgttcattcgtatttctcctctagacaagcgaggggaaactccctcgctatagtggtggattcagtgaatcaaataatgtcgtttgttgattaaaagggaaggtcatcatctgaaatatcaattgcagaactacctgcaaatggatcgtttgaatgttgctgtgcaaatgtgtttttatttgcttcattactgataggacgttccacgccgttaggcttacttccttcttcatcaagtttgttataagctttcacagataaattccatctgtcgttataatcactatgtttccaatcaacagtaatatttaatgttttaccttttgcggcagtgactaattgttgaatactatcaattgctgttccgtccggtactccaattgctgttaaaatcgtattaaatcgtttagtagaaaattcaatatcgttgttatcccacacaatattgtcgtaaagaatttttccacctttatatttgccgtcgatcacttcataattgaagacagccatatcattatttgtttcttttgtttttttgcactcagaatcaggaagaatttttacattgtaacttcctgcttcttttactgatttgcctaaaacattttgtgaatctactacaaatagtgccatattaaattccttcttcctgatgattatttattagttcctttgcttcgataagcttgcgatcatcgattctattttttgcatgattcccgttttctggatttaaatcaatcaaacgtttatcatcatcaatatagatacgaccgactaaatcaaacattgatgtaaaagcattaaaggtcttttcgttcatatctggactaaaacgtcctttgccatctaatccgctagcaccattgtcaacttggtgtgcagttgcataaatagttttgttgctctctcttaattttgttcctaattgtctgaaccatagttgcaatttctgataattttgacgtccgtctcgtgaagctccgtcaatattttctagtactaaattttgtaaggcagtcatgttgtctaagataatgacttcgtattctggtttgctcaatgctcctagtacccacttatctattaatgattggatattaggcgcatctccactttctaactgaacaacagagatatctttttccccaattaatacgttcgttgataaatcaaaactaaaaagtattttatttccttcaaactgtttagctagtgaagtttttcctgtacctccatcaccgtaaataaaatacatattcgcttgttttggtactgttccatttggatagaatttcatacctgcttcaccttcacttttacttctggctctttgataccaactgttagattcggaatataacaaccattctcatctattactcgaagatcatccgttagttgaaacacaccgtcagcaatcaacttcttgatgtctagttgctttggtttgtattcagttgattctttgaccaattcaggatgttcgtttcgaaggtattgaataaattgttctttctcttcttttactttggatggttgtaatttaaaatgcgatggcttacgcaaatctacaggcttcatcgtcaaaacaaagcttttggtttcgactaattctgcattgcccatcaactgtctttggataactactgcttcatcaatttctttttgtaaatctgcacatacacgattctttctttccgttatctgtgcaatttcaatatcgtattgattaagccgatgtttctttgcttgttctaattcctcgatttttttcgtgatccattccaaatcatatccttcaaaatgactcatcttcgtcctcctcatcgattggtgcttcatatggtggtttagcataatcaggatcagttaaatagttgtcaagatttgctaactcgttcatatttcccctcttttcctcttgctagcacgcaaagcacaagcatggcaattgcgaataacaagccaaagattacgtaccttttcgctacaatcactaacgtgaaaaataaaataatgaatagatcaattgttttttcgttcatgtgtgataacatcctttactgtaattcttcttctgaaaaagaacttttgttgctcaaatacgttgatggcgtactcgtagttgtcttctgttaagtcgttgatacgctcaatttctaaacaagcttttacagcttcataaatagcattcttttgatttagaataattcttcgattgtctcgttgattttcaagccatgcctcgactaccttaccgaatttatatccgtaattgattctcggtttatttcgttcagctaattgcttttcaacctcttcggcaatacgtttactcaattcttctgtcgtcattgtcaccatttctgccattgttgttcctccgttatcatggtatactttagctaaaatgatttttaaaaagtgcatcaacacttgtgccgagtatttcggctagtttgaatgcggtactcaagcttggtaggcgtgtaccgtattcaaatctttggtatgaagttagcgttattcctaatttttttgctacttcatgttgctttagacctgcattttcgcgggctttttttagtttttcgttattcaaatcacatcccactttctttattgattacatccaattaggttgtaacctaattttattatacatccacattggttgtagtcaagtatttttattttggaggttttctcatggaaacaaacattcctgacagattaaaacaacttagggaaacagccaatttgactcaatcagatatggcagaaatacttgatgtaaaactgcaaagttatcaacgtttcgaatacggtagtagacgccccagtctcgatgtattaatcgccctcgccgactacttcgatgtatcgcttgattatttagtcggtagaacagacgagaaatgatcgcttaggcggtctttttttgtttccgcagtctttgatataatcttcttatcaggatgacagactgaaatatctgataaggaggtaaagctatggactatgataatttttatcaagttgaaagttttctagttactcgcaaagaagaaaaatatgtcaacgaactattaaaatttggatggaaattgatttctgtgattcagtacaaagatgactatgacgcatatggtaaatatgtgttaggtgctgacaaaaatacttttgaaaaacgtaattttcaaatgattcttaatgaagaaaacgaacaagatccattgccattttagtttcttgcttcaggatgtttcatctcaaaattctttaattgctccttgctatttctgatagcttggagctctttttttatttcttcttgcgattcaataattttttgctgttgcttaagaagctcattgagtgctaccatttgtaattcttccatttgactacctccgtttctaagtgataaacttaacttactagttatgattttttaccaattagcgaccctcatcgctagttggtctttttttacttctcgccacttcttctggcgttcacgccattgttcccctaacaatctaggtttcatttcttcgtggtattcctgatttagttttcgcatcaagtgttgatgctcttgtaaggtcatttgatccctccttcgtttctcaccgtcaccacctccggaaagaggagttgcccatgccaacgtgtatatgcgaacttgatttttaaggagaaaactcgcaactcctcttttcggaagtggtgcgtgtgtgatataatattattgttctatggtgcccactacttgcttgccggctgtgtgggcttttctttttgttcaattatggttgccaccacagtaactccccaatgtctagaacgtattctagccatttcatctgctaatctttgaagattaggtgtgccattcaaagtgatttttggcttgttactcacaatctcacatcctacactgttgattttcgttcatttcttttgctaaaatttcattatcagtgagtggtccactgaaataactgataaggcggtgataaatatggggatgactgataaagagatcgctttggagattacgaagtcttatttaaatcatttatctgatagggctagaagcaacaatattaacgaatctcatgctacagcccaaaatgtttgcaacatgtacaaagtattttatgatgtggtgtcttctgtaggaaagtcttctagtggtaaagaatagttatttttttcaatacaaaagttaacatcatacttttcatttagaacttctaggtcggctaggagttctttggcgttttcaatactttctacttgtgctgatacttcaattatttgtttcttcatccttctcacctcacgctggttgattaacgttcgcatactttcggtcaatccctaaaaagtctgcgattttcaacttgtaaaagtccgctttattgtcttgttatccacctcttgataaaattagtttgaaagcgaggtgaataataaatggataatatccctaaaaacttaagtaaagaagaacttgagcttgtaactgatatgctttatactttacgagattttctaaaaaagaaatctattagaagtaattctaaaacaggtcaaatgatgaatgaattagagatagaacttcagaacatagctcttaaacatttattcaatcagcgcagataactcgttggcagctttaactctttcatccaagccttcatgtcgatttcctcgtaatatacttgataattctttttctctgcctttggtaaatgaatcttgaagtctttttttaaagacttctttattttcgattttttgagaagttaaattatcttgaaaacttctatcaacaatttctttgattttttgccactcataaaatttcaattctgacaagacattaaacaactcgtttttttgtttttccacttgcttcacctcctacattgattgctcactcacctcttggtagaattattaatatagaaaggcggtgatttttttatggctattgctaatacagatacttttgctcttgctgtcgttcaatcatctgatccaaaattaacagttgaagaaaaaatctctctttacattgaagcaagagacaaagcaaaagaatacaataaaaaacatcctaataaaggagtcaaccttaaaaaaatttaaccgtaccaatgtgttaaaacctgtaaaagctctgcaatggaagccgccatttcagggcttttatcatctaaatcaatcaattcagaggtataagctattgctttttcatataattcgtccatctccctacacctcctacgctggttgttggttaccttcaagtcgcacaaacgcgactttttgctaaaaaaaatttcaactgcttcagaatctgttaatggaacttcttctttaatttttttagcttcagctatagtaaaatctccaccgtttttcatttttctatagaatgtacttctgttaattccgattgaatcggcaactgcttgttgagtagttccacgctcaactattaatccttttaatttagctacatcaatcataaataacacctctctttttgtcgcatttatgcgacttgatattttaaatatacatcaatatctcaaaacagtcaacacaaaagttgcatttttgcgattgtttttgttgcaaatttgcaacataatttatataatagtgattggaggtgatggaatgactgtaggagaaaaaatgaagtttagaagaaaagaactaaaaataagtgcggatgaaatagcaaaagccttaggtgtttccagatcaaccatatttagatatgaaaaaggggaaatagaaaaactaccaacagaaaatttacgaaaaatagccgaagttttgaaaacaactcctgaagaattaatgggatggactgaaactgaaaataatttttctatagtgtctatttacaaccaacttgtttcacctcgacaacaaaaagtatatgactttgctaaacatgagttagaagaacagcaagagtcagaacgaagaaataaaattcagtctcttcaaaaatatagagaaatgaaagagcaaaaagaagaatttgccgatatagaatggtacggatgtgcttcagcaggtactggagaattcatgtttgataataaagaagtgatttcacttcctaaaaaacaaattcctttagaagctgatttttgcttaactgtcaatggtgactctatggaaccattaattcaccatcatgattatattttcgtttctaaacaagatactttatttaacggaaacattggcgttgttatcgtagacggagaagcattcattaaaaaagttttttttgaaaatgataaagctcgtttacaatcatttaataaaaaatataaagacattattgttgatgattctaacgattttaggattattggcaaagtggttttataaaaaaagaaccacctaccaatttggctaggtggtttttatataaatatttttaaagtaaggagttttagttttatgaaaaaaattattattagtatatcaattatcgcaattattatttttggaggaattttctactacacacaagtgaaacgtccacatgacgaagccgtggagaaatatgaacaagttatttcagaacgaaaaaaacaaaataacaatttacaagatttaattaaccaatctgaaaatattattaaaggaaaaaacaaaccgtataagcaagaaactttcgattctttaaaaaaagaaatagatattgctaaaaaagaattaattaatatacctaacataccttcaaaaactaaagatattttagaagatgttgaaaaattcacacatccattcaactattcagatattgaaagtaagttaaaagaaaaaatggaagctgcacaaaatagcataaaacaattaaaacaagtaacagctccttcacaagatttcattttaaatagaattaaagaagttaagaatatcgatgctgtcgaacctgcaacagaagcaaacgatccgaacgaactcctcaataaagcaggaggatatactgcagctattttctttagttctcctttagtaaatcaatctgaagtctacggtgaatcaattattgataaaggtacagacggaggaggatgcatagaagtatatgctaatacagaagatgcagaaaaaagagataaatatttagcagcatttgatggaggatctctcagcccaggttctcataaagttttaggtactttagttattcgtacatcagcaaagttgacagctactcaacaaaatgaattaactaatgacattatcaatagtttaattaagttataaaagtttagccttcgggcttttcttttacaatcaataagaacgtacattcgaaaggagataacatgaaacgagtagcattatatatgagagtatcaactgaacaacaagccaaacatggagatagtcttagagaacaaaaagaaaccctctatgaatatatcgaacaacacaaggatttgaaagtagttaatgaatatgtagacggtggtatttctggtcaaaaaataaatcgtgatgaatttcaaaaactattacaagatgtaaaagaaaataaaatagatctaattttatttacaaaattagatagatggtttagaaatctacgacattatttaaacactcaagaaattttagaaaaacacaacgtttcttggaatgctgtttcgcaacaatattatgatacaactacagcgtatggcagaactttcattgcacaagtaatgagttttgctgaattggaagcccaaattgattcggaacgcatcaaagctgttatggcaaataaaattgcacaaggtgaagtagtaagcgggaaaactccgttaggctactctatagaaaataagaaattagtaataaatgatgatgctcctatcgtgatagatatattcaactactttctttctagtggtagtttaagaaaaactgtttattatttaggctctcagtatggaatcgttagagattatcaaagtgttaaaaatatgttgacgaacaaaaaatacattggtgaattaagaaataataaaaattactgtcctcctattattgataaaaaacttttttatgctgttcaaaaagcattacctaaaaatttaaaaacaaatgcaaaacgcgattacatttttaaaggtttattaaaatgttctgactgtcagggatcagtagctggtcaaactattaaagcaagatataagaaaaaagacggtacagaatcaatatacgaaagaacttgttatagatgtgtaaaacgaagaaataataaattacgttgtacaaataagcgcgctttttacgaaaaaaatttagaacgttatatttttgaagctactaaacaaaaatttgaacaaatacaaataaactattcaaaaaaacaaccaaagattattaaaaagaaaaatagtaagaaaaatattgagaataaattagatagattgaagaaagcctacttgaatgaagttatagacttagaggaatacaaaaaagatcgagaagctttaatgaaagaattaaatgaaattgaagtagagccagctaaaatagatataaaaaatgtcgaatttattctatcaaaagaattcgatgaaatttataaagaatcttctaaagaagaaaaaaatgcattatggcgttcaattatcgataacataatagtatttccagatggcaatataacagtaaatttccttttataatttatgtgtactaacttatatattccagatggatgattatgaactaaaataattctcgctgcagaatatcgaacagcataatggaacacttctcttggatgtgcgatcgtttgatccagggaaccaataaatagcgtttttttcaacaatacttgattcttagtatccaaataaatacaaatcaaatgttcttgtttgtgatcctttaattctatgattaattgatgcgctaattcatagctggcatggatcgtgggttgtaccgctacatgctgtgtttggattctttttcctagctcgatcagtgctttgatttcaagagccttaacctgaccaattcctcgtattttttccagctcagacagcgttgcctgtcttaacagtgcaagtccaccaaatgttttcaacaaattacctgctagttccaagacattatagggatgctgtcccgtgcgtaataaaatagcaagtaattcttgatcagagagtgctttctctccgtaaagcaacattcgctcccttggaagtgaggttgctggcacagcatccagcaaatttttttccataaaatcccccctttcttcttctcactaataagatacgaaaaaaggggggagctatttttatttttttagatatcctggtacttcgtgtagagaagataaaactgctaacgttttttgttgcaagtcttctgaaggagccaacaaatctgggatcatgatcactgggatctccgcacttgctgctgcaagtatcccgtttttagaatcttccagaaccaatgtttcttgttttttcgttcctagatattcatgggcaagcaaaaagatttctggatcaggtttagcacgtttgacattttctgctgaaacaatcgtttcaaaatagtttgtcagttggttcttttccaataatagctcaataatatgacgttggttactagaagcgacaactttaggtattcggtgttcttctaaaaagtccagtaattcgattactcctggttttaattgcactgcacctaaggaaaaccgtctgatcgtttcttcataagcatcattaatgaatttttgaacattgtttttcccaaaacttgcaaagatctgatgataatttgcccaaacctcttcatctgatacacctagatattttaaatacaattctttgtcgtaaggaaagcccatttgatcagcaaccatttgcgaggcttcatagtagacgatttctgtgtcaaagagtaacccatccatgtcaaaaatgacagctttataattcat

SEQ ID NO: 3 - protein, 9 aa, Enterococcus hirae
SAFPYEQEL

SEQ ID NO: 4 - protein, 9 aa, Enterococcus hirae
YNYSKSYPV

SEQ ID NO: 5 - protein, 9 aa, Enterococcus hirae
VSFSHYRPG

SEQ ID NO: 6 - protein, 9 aa, Enterococcus hirae
VTFLGYNAF

SEQ ID NO: 7 - protein, 9 aa, Enterococcus hirae
TVYTFHVNI

SEQ ID NO: 8 - protein, 9 aa, Enterococcus hirae
TSYSPLFLL

SEQ ID NO: 9 - protein, 9 aa, Enterococcus hirae
TNYIYPNIL

SEQ ID NO: 10 - protein, 9 aa, Enterococcus hirae
VVPILFLGL

SEQ ID NO: 11 - protein, 9 aa, Enterococcus hirae
KNYKAYVEL

SEQ ID NO: 12 - protein, 9 aa, Enterococcus hirae
SAMKYGIPL

SEQ ID NO: 13 - protein, 9 aa, Enterococcus hirae
TSLARFANI

SEQ ID NO: 14 - protein, 9 aa, Enterococcus hirae
AMIEFIQGL

SEQ ID NO: 15 - protein, 9 aa, Enterococcus hirae
VAITFGGPL

SEQ ID NO: 16 - protein, 9 aa, Enterococcus hirae
VSTNHYGLL

SEQ ID NO: 17 - protein, 9 aa, Enterococcus hirae
VMFGLFITI

SEQ ID NO: 18 - protein, 9 aa, Enterococcus hirae
TVFSLVSLL

SEQ ID NO: 19 - protein, 9 aa, Enterococcus hirae
SIYNLEKPL

SEQ ID NO: 20 - protein, 9 aa, Enterococcus hirae
YTIIRYGNL

SEQ ID NO: 21 - protein, 9 aa, Enterococcus hirae
SNGLLYTPM

SEQ ID NO: 22 - protein, 9 aa, Enterococcus hirae
NNYHYVGGL

SEQ ID NO: 23 - protein, 9 aa, Enterococcus hirae
SMFLNCNNL

SEQ ID NO: 24 - protein, 9 aa, Enterococcus hirae
IAFQGYSSL

SEQ ID NO: 25 - protein, 9 aa, Enterococcus hirae
QVTNFFNMF

SEQ ID NO: 26 - protein, 9 aa, Enterococcus hirae
IMLGLFMTM

SEQ ID NO: 27 - protein, 9 aa, Enterococcus hirae
INAKFSSQL

SEQ ID NO: 28 - protein, 9 aa, Enterococcus hirae
YIYNHYKDM

SEQ ID NO: 29 - protein, 9 aa, Enterococcus hirae
YVYGKSRTM

SEQ ID NO: 30 - protein, 9 aa, Enterococcus hirae
IAFLSYKLF

SEQ ID NO: 31 - protein, 9 aa, Enterococcus hirae
IMYEYMYPV

SEQ ID NO: 32 - protein, 9 aa, Enterococcus hirae
SSMEYFLKV

SEQ ID NO: 33 - protein, 9 aa, Enterococcus hirae
ISFFQENQL

SEQ ID NO: 34 - protein, 9 aa, Enterococcus hirae
TNLLFMTSL

SEQ ID NO: 35 - protein, 9 aa, Enterococcus hirae
KIFSIFMLL

SEQ ID NO: 36 - protein, 9 aa, Enterococcus hirae
LNIFKFNRF

SEQ ID NO: 37 - protein, 9 aa, Enterococcus hirae
MTYDYRGGF

SEQ ID NO: 38 - protein, 9 aa, Enterococcus hirae
PSYMFRTSF

SEQ ID NO: 39 - protein, 9 aa, Enterococcus hirae
QSYTYYMTA

SEQ ID NO: 40 - protein, 9 aa, Enterococcus hirae
ITFSHYEPT

SEQ ID NO: 41 - protein, 9 aa, Enterococcus hirae
MSFTFFSST

SEQ ID NO: 42 - protein, 9 aa, Enterococcus hirae
IAFQNFVNL

SEQ ID NO: 43 - protein, 9 aa, Enterococcus hirae
SMFIAFQNF

SEQ ID NO: 44 - protein, 9 aa, Enterococcus hirae
LNYDYGNRI

SEQ ID NO: 45 - protein, 9 aa, Enterococcus hirae
AGICFFTGV

SEQ ID NO: 46 - protein, 9 aa, Enterococcus hirae
VEYTYFPTL

SEQ ID NO: 47 - protein, 9 aa, Enterococcus hirae
AAYVFEMNF

SEQ ID NO: 48 - protein, 9 aa, Enterococcus hirae
EMYRKLSTL

SEQ ID NO: 49 - protein, 9 aa, Enterococcus hirae
YNYGYKSVL

SEQ ID NO: 50 - protein, 9 aa, Enterococcus hirae
VIHELYNSL

SEQ ID NO: 51 - protein, 9 aa, Enterococcus hirae
TNYVKLRPL

SEQ ID NO: 52 - protein, 9 aa, Enterococcus hirae
QAVNHFTGI

SEQ ID NO: 53 - protein, 9 aa, Enterococcus hirae
YTDYSNQLK

SEQ ID NO: 54 - protein, 9 aa, Enterococcus hirae
AMIEFIQGL

SEQ ID NO: 55 - protein, 9 aa, Enterococcus hirae
KMVEILEEI

SEQ ID NO: 56 - protein, 9 aa, Enterococcus hirae
RLLKYDVGV

SEQ ID NO: 57 - protein, 9 aa, Enterococcus hirae
TLVGVTFAI

SEQ ID NO: 58 - protein, 9 aa, Enterococcus hirae
AMQNLVAAV

SEQ ID NO: 59 - protein, 9 aa, Enterococcus hirae
AIMAIANGV

SEQ ID NO: 60 - protein, 9 aa, Enterococcus hirae
AMSMNMEEV

SEQ ID NO: 61 - protein, 9 aa, Enterococcus hirae
KVFGKMTSV

SEQ ID NO: 62 - protein, 9 aa, Enterococcus hirae
LLGIYQSYV

SEQ ID NO: 63 - protein, 9 aa, Enterococcus hirae
KLAKFASVV

SEQ ID NO: 64 - protein, 9 aa, Enterococcus hirae
KLWANMSKA

SEQ ID NO: 65 - protein, 9 aa, Enterococcus hirae
MLSNPITAI

SEQ ID NO: 66 - protein, 9 aa, Enterococcus hirae
ILVAITTTI

SEQ ID NO: 67 - protein, 9 aa, Enterococcus hirae
KMAALAASA

SEQ ID NO: 68 - protein, 9 aa, Enterococcus hirae
AMLSNPITA

SEQ ID NO: 69 - protein, 9 aa, Enterococcus hirae
NMAEAFASA

SEQ ID NO: 70 - protein, 9 aa, Enterococcus hirae
TMFSDSALK

SEQ ID NO: 71 - protein, 9 aa, Enterococcus hirae
LLTRFTTLK

SEQ ID NO: 72 - protein, 9 aa, Enterococcus hirae
KTAFSGIVK

SEQ ID NO: 73 - protein, 9 aa, Enterococcus hirae
KTISTMFEK

SEQ ID NO: 74 - protein, 9 aa, Enterococcus hirae
VFGKMTSVF

SEQ ID NO: 75 - protein, 9 aa, Enterococcus hirae
AYFNHTLDL

SEQ ID NO: 76 - protein, 9 aa, Enterococcus hirae
AWKSNFMNI

SEQ ID NO: 77 - protein, 9 aa, Enterococcus hirae
RYGTTESQL

SEQ ID NO: 78 - protein, 9 aa, Enterococcus hirae
SYVNNGASI

SEQ ID NO: 79 - protein, 9 aa, Enterococcus hirae
KYKSNLAGL

SEQ ID NO: 80 - protein, 9 aa, Enterococcus hirae
VFGKMTSVF

SEQ ID NO: 81 - protein, 9 aa, Enterococcus hirae
AFSGIVKSF

SEQ ID NO: 82 - protein, 9 aa, Enterococcus hirae
VYTDYSNQL

SEQ ID NO: 83 - protein, 9 aa, Enterococcus hirae
AFQNQITQL

SEQ ID NO: 84 - protein, 9 aa, Enterococcus hirae
VINPIGSLR

SEQ ID NO: 85 - protein, 9 aa, Enterococcus hirae
KAKIKSPSR

SEQ ID NO: 86 - protein, 9 aa, Enterococcus hirae
KTISTMFEK

SEQ ID NO: 87 - protein, 9 aa, Enterococcus hirae
ASKAGGGFR

SEQ ID NO: 88 - protein, 9 aa, Enterococcus hirae
RTFAATGIR

SEQ ID NO: 89 - protein, 9 aa, Enterococcus hirae
GNKVTNFFR

SEQ ID NO: 90 - protein, 9 aa, Enterococcus hirae
ITGSRLIKR

SEQ ID NO: 91 - protein, 9 aa, Enterococcus hirae
DVFEGAVKR

SEQ ID NO: 92 - protein, 9 aa, Enterococcus hirae
EAFASADPK

SEQ ID NO: 93 - protein, 9 aa, Enterococcus hirae
DVFEGAVKR

SEQ ID NO: 94 - protein, 9 aa, Enterococcus hirae
TMFSDSALK

SEQ ID NO: 95 - protein, 9 aa, Enterococcus hirae
ESAFTGVKK

SEQ ID NO: 96 - protein, 9 aa, Enterococcus hirae
TSVAVQSAK

SEQ ID NO: 97 - protein, 9 aa, Enterococcus hirae
DTAATSLAR

SEQ ID NO: 98 - protein, 9 aa, Enterococcus hirae
MIEFIQGLK

SEQ ID NO: 99 - protein, 9 aa, Enterococcus hirae
MALLAGMLR

SEQ ID NO: 100 - protein, 9 aa, Enterococcus hirae
RTFAATGIR

SEQ ID NO: 101 - protein, 9 aa, Enterococcus hirae
FSGIVKSFK

SEQ ID NO: 102 - protein, 9 aa, Enterococcus hirae
EAGGSAFSR

SEQ ID NO: 103 - protein, 9 aa, Enterococcus hirae
TSVGSNMAK

SEQ ID NO: 104 - protein, 9 aa, Enterococcus hirae
KTISTMFEK

SEQ ID NO: 105 - protein, 9 aa, Enterococcus hirae
YTDYSNQLK

SEQ ID NO: 106 - protein, 9 aa, Enterococcus hirae
MVEILEEIR

SEQ ID NO: 107 - protein, 9 aa, Enterococcus hirae
VINPIGSLR

SEQ ID NO: 108 - protein, 9 aa, Enterococcus hirae
EDFANVTGR

SEQ ID NO: 109 - protein, 9 aa, Enterococcus hirae
IAGFVDGLR

SEQ ID NO: 110 - protein, 9 aa, Enterococcus hirae
TPMGKMVEI

SEQ ID NO: 111 - protein, 9 aa, Enterococcus hirae
NLLTRFTTL

SEQ ID NO: 112 - protein, 9 aa, Enterococcus hirae
RLIKRSNAI

SEQ ID NO: 113 - protein, 9 aa, Enterococcus hirae
ARFANITQM

SEQ ID NO: 114 - protein, 9 aa, Enterococcus hirae
FRTFAATGI

SEQ ID NO: 115 - protein, 9 aa, Enterococcus hirae
LRAIITVGK

SEQ ID NO: 116 - protein, 9 aa, Enterococcus hirae
ARFANITQM

SEQ ID NO: 117 - protein, 9 aa, Enterococcus hirae
QQMALLAGM

SEQ ID NO: 118 - protein, 9 aa, Enterococcus hirae
RLIKRSNAI

SEQ ID NO: 119 - protein, 9 aa, Enterococcus hirae
NPSQAMIEF

SEQ ID NO: 120 - protein, 9 aa, Enterococcus hirae
FANASTEYM

SEQ ID NO: 121 - protein, 9 aa, Enterococcus hirae
EAEAGGSAF

SEQ ID NO: 122 - protein, 9 aa, Enterococcus hirae
MAALAASAG

SEQ ID NO: 123 - protein, 9 aa, Enterococcus hirae
FAAALSSVG

SEQ ID NO: 124 - protein, 9 aa, Enterococcus hirae
LAASAGPVL

SEQ ID NO: 125 - protein, 9 aa, Enterococcus hirae
AAVKWESAF

SEQ ID NO: 126 - protein, 9 aa, Enterococcus hirae
SKADIVNTL

SEQ ID NO: 127 - protein, 9 aa, Enterococcus hirae
IKNGSSSAL

SEQ ID NO: 128 - protein, 9 aa, Enterococcus hirae
NKLNNNQAL

SEQ ID NO: 129 - protein, 9 aa, Enterococcus hirae
VEAYFNHTL

SEQ ID NO: 130 - protein, 9 aa, Enterococcus hirae
TEVRLRDSL

SEQ ID NO: 131 - protein, 9 aa, Enterococcus hirae
SELEQGAQL

SEQ ID NO: 132 - protein, 9 aa, Enterococcus hirae
TEVRLRDSL

SEQ ID NO: 133 - protein, 9 aa, Enterococcus hirae
AEAAGQLGI

SEQ ID NO: 134 - protein, 9 aa, Enterococcus hirae
KGLGNIFKW

SEQ ID NO: 135 - protein, 9 aa, Enterococcus hirae
IANGVKGLW

SEQ ID NO: 136 - protein, 9 aa, Enterococcus hirae
KAGNIDSKW

SEQ ID NO: 137 - protein, 9 aa, Enterococcus hirae
KSNPSQAMI

SEQ ID NO: 138 - protein, 9 aa, Enterococcus hirae
RSFSASLQL

SEQ ID NO: 139 - protein, 9 aa, Enterococcus hirae
RAANASDVF

SEQ ID NO: 140 - protein, 9 aa, Enterococcus hirae
STAGVEAYF

SEQ ID NO: 141 - protein, 9 aa, Enterococcus hirae
LSNPITAIL

SEQ ID NO: 142 - protein, 9 aa, Enterococcus hirae
LSNSKLAKF

SEQ ID NO: 143 - protein, 9 aa, Enterococcus hirae
FANASTEYM

SEQ ID NO: 144 - protein, 9 aa, Enterococcus hirae
FKSNPSQAM

SEQ ID NO: 145 - protein, 9 aa, Enterococcus hirae
LAASAGPVL

SEQ ID NO: 146 - protein, 9 aa, Enterococcus hirae
EASKASGSL

SEQ ID NO: 147 - protein, 9 aa, Enterococcus hirae
VAITFGGPL

SEQ ID NO: 148 - protein, 9 aa, Enterococcus hirae
SAISAAKPM

SEQ ID NO: 149 - protein, 9 aa, Enterococcus hirae
EAFNENTAL

SEQ ID NO: 150 - protein, 9 aa, Enterococcus hirae
SANNAGREL

SEQ ID NO: 151 - protein, 9 aa, Enterococcus hirae
AAGKSGTVL

SEQ ID NO: 152 - protein, 9 aa, Enterococcus hirae
KAAKSTEEL

SEQ ID NO: 153 - protein, 9 aa, Enterococcus hirae
FASVVINPI

SEQ ID NO: 154 - protein, 9 aa, Enterococcus hirae
FAATGIRSI

SEQ ID NO: 155 - protein, 9 aa, Enterococcus hirae
RAANASDVF

SEQ ID NO: 156 - protein, 9 aa, Enterococcus hirae
ASIDQQMAL

SEQ ID NO: 157 - protein, 9 aa, Enterococcus hirae
AAKPMIEAL

SEQ ID NO: 158 - protein, 9 aa, Enterococcus hirae
NAKQKGAEL

SEQ ID NO: 159 - protein, 9 aa, Enterococcus hirae
TAVNAIMAI

SEQ ID NO: 160 - protein, 9 aa, Enterococcus hirae
SADPKTQEF

SEQ ID NO: 161 - protein, 9 aa, Enterococcus hirae
NASDIPSNL

SEQ ID NO: 162 - protein, 9 aa, Enterococcus hirae
SADTAATSL

SEQ ID NO: 163 - protein, 9 aa, Enterococcus hirae
FASADPKTQ

SEQ ID NO: 164 - protein, 9 aa, Enterococcus hirae
EAEAGGSAF

SEQ ID NO: 165 - protein, 9 aa, Enterococcus hirae
FVSKYKSNL

SEQ ID NO: 166 - protein, 9 aa, Enterococcus hirae
AAVKWESAF

SEQ ID NO: 167 - protein, 9 aa, Enterococcus hirae
IASLTGAML

SEQ ID NO: 168 - protein, 9 aa, Enterococcus hirae
SAAGKSGTV

SEQ ID NO: 169 - protein, 9 aa, Enterococcus hirae
FGGPLVAAL

SEQ ID NO: 170 - protein, 9 aa, Enterococcus hirae
IKNGSSSAL

SEQ ID NO: 171 - protein, 9 aa, Enterococcus hirae
SADPKTQEF

SEQ ID NO: 172 - protein, 9 aa, Enterococcus hirae
MVDSNGKVI

SEQ ID NO: 173 - protein, 9 aa, Enterococcus hirae
SADTAATSL

SEQ ID NO: 174 - protein, 9 aa, Enterococcus hirae
LKDTIVGLF

SEQ ID NO: 175 - protein, 9 aa, Enterococcus hirae
ARFANITQM

SEQ ID NO: 176 - protein, 9 aa, Enterococcus hirae
ARFANITQM

SEQ ID NO: 177 - protein, 9 aa, Enterococcus hirae
FAATGIRSI

SEQ ID NO: 178 - protein, 9 aa, Enterococcus hirae
FASVVINPI

SEQ ID NO: 179 - protein, 9 aa, Enterococcus hirae
FVEAGVNKL

SEQ ID NO: 180 - protein, 9 aa, Enterococcus hirae
FANASTEYM

SEQ ID NO: 181 - protein, 9 aa, Enterococcus hirae
VVMDTGQVV

SEQ ID NO: 182 - protein, 9 aa, Enterococcus hirae
KVFGKMTSV

SEQ ID NO: 183 - protein, 9 aa, Enterococcus hirae
AYFNHTLDL

SEQ ID NO: 184 - protein, 9 aa, Enterococcus hirae
SYVNNGASI

SEQ ID NO: 185 - protein, 9 aa, Enterococcus hirae
VYTDYSNQL

SEQ ID NO: 186 - protein, 9 aa, Enterococcus hirae
FFRSFSASL

SEQ ID NO: 187 - protein, 9 aa, Enterococcus hirae
RSFSASLQL

SEQ ID NO: 188 - protein, 9 aa, human
KLQKFASTV

SEQ ID NO: 189 - protein, 9 aa, mouse
GSLARFRNI

SEQ ID NO: 190 - protein, 9 aa, artificial sequence
  mutated peptide
GSFARFRNI

SEQ ID NO: 191 - DNA, 20 bp, Artificial Sequence
  primer
actgcagccgtaaaatggga

SEQ ID NO: 192 - DNA, 20 bp, Artificial Sequence
  primer
tccgtatcgtttgccagctt

SEQ ID NO: 193 - DNA, 92 bp, Artificial Sequence
  primer
caataaaaaatcagacctaagactgatgacaaaaagagcaaattttgataaaatagtattagaattaaattaaaaagggaggccaaatatag

SEQ ID NO: 194 - DNA, 100 bp, Artificial Sequence
  primer
gatcctatatttggcctccctttttaatttaattctaatactattttatcaaaatttgctctttttgtcatcagtcttaggtctgattttttattgcatg

SEQ ID NO: 195 - DNA, 36 bp, Artificial Sequence
  primer
tccggatccatggcacaaagtaaaacagtcaaagcg

SEQ ID NO: 196 - DNA, 66 bp, Artificial Sequence
  primer
caggaattcttacttgtcgtcatcgtctttgtagtcacgtagtaaactatcacgtaatcgaacttc

SEQ ID NO: 197 - DNA, 35 bp, Artificial Sequence
  primer
aacgagctaaggcagtagcagctgtatctgcagac

SEQ ID NO: 198 - DNA, 35 bp, Artificial Sequence
  primer
gtctgcagatacagctgctactgccttagctcgtt

SEQ ID NO: 199 - DNA, 38 bp, Artificial Sequence
  primer
attagcaaaacgagcgaaggaagtagcagctgtatctg

SEQ ID NO: 200 - DNA, 38 bp, Artificial Sequence
  primer
cagatacagctgctacttccttcgctcgttttgctaat

SEQ ID NO: 201 - DNA, 27 bp, Artificial Sequence
  primer
cttggatccatggtgagcaagggcgag

SEQ ID NO: 202 - DNA, 31 bp, Artificial Sequence
  primer
caggaattcctacataattacacactttgtc

SEQ ID NO: 203 - DNA, 23 bp, Artificial Sequence
  primer
cccagtcacgacgttgtaaaacg

SEQ ID NO: 204 - DNA, 24 bp, Artificial Sequence
  primer
gagcggataacaatttcacacagg

SEQ ID NO: 205 - DNA, 20 bp, Artificial Sequence
  gRNA
agatattgcggaaacgagcc

SEQ ID NO: 206 - DNA, 20 bp, Artificial Sequence
  primer
ctcagggacccttttcacga

SEQ ID NO: 207 - DNA, 20 bp, Artificial Sequence
  primer
cccactccctgttctacaca

SEQ ID NO: 208 - DNA, 21 bp, Artificial Sequence
  primer
ggacccttttcacgattcagg

SEQ ID NO: 209 - protein, 9 aa, artificial sequence
  peptide with variable positions
  X=AorQ (3)..(3)
  X=VorT (8)..(8)
KLXKFASXV

SEQ ID NO: 210 - protein, 9 aa, Artificial Sequence
  hybrid
KLAKFASTV

SEQ ID NO: 211 - protein, 9 aa, artificial sequence
  hybrid
KLQKFASVV